European Patent Application EP 4 810 067 A1, published September 23, 2026. Title: 一种生物素或亲和素标记脂肪体及其制备方法、纳米载体系统. Applicant: 维康平生（北京）生物科技有限公司. The sequence listing filed with the application follows.

SEQUENCE LISTING (3 sequences)

SEQ ID NO: 1 - protein, 371 aa, synthetic construct
MVSKGEELFTGVVPILVELDGDVNGHKFSVSGEGEGDATYGKLTLKFICTTGKLPVPWPTLVTTLTYGVQCFSRYPDHMKQHDFFKSAMPEGYVQERTIFFKDDGNYKTRAEVKFEGDTLVNRIELKGIDFKEDGNILGHKLEYNYNSHNVYIMADKQKNGIKVNFKIRHNIEDGSVQLADHYQQNTPIGDGPVLLPDNHYLSTQSALSKDPNEKRDHMVLLEFVTAAGITLGMDELYKGGGSARKCSLTGKWTNDLGSNMTIGAVNSRGEFTGTYITAVTATSNEIKESPLHGTQNTINKRTQPTFGFTVNWKFSESTTVFTGQCFIDRNGKEVLKTMWLLRSSVNDIGDDWKATRVGINIFTRLRTQKE

SEQ ID NO: 2 - DNA, 1119 bp, synthetic construct
  source 1..1119: mol_type = other DNA
atggtgagcaagggcgaggagctgttcaccggggtggtgcccatcctggtcgagctggacggcgacgtaaacggccacaagttcagcgtgtccggcgagggcgagggcgatgccacctacggcaagctgaccctgaagttcatctgcaccaccggcaagctgcccgtgccctggcccaccctcgtgaccaccctgacctacggcgtgcagtgcttcagccgctaccccgaccacatgaagcagcacgacttcttcaagtccgccatgcccgaaggctacgtccaggagcgcaccatcttcttcaaggacgacggcaactacaagacccgcgccgaggtgaagttcgagggcgacaccctggtgaaccgcatcgagctgaagggcatcgacttcaaggaggacggcaacatcctggggcacaagctggagtacaactacaacagccacaacgtctatatcatggccgacaagcagaagaacggcatcaaggtgaacttcaagatccgccacaacatcgaggacggcagcgtgcagctcgccgaccactaccagcagaacacccccatcggcgacggccccgtgctgctgcccgacaaccactacctgagcacccagtccgccctgagcaaagaccccaacgagaagcgcgatcacatggtcctgctggagttcgtgaccgccgccgggatcactctcggcatggacgagctgtacaagggaggaggaagcgccaggaagtgcagcctgaccggcaagtggacaaacgatctgggcagcaacatgaccatcggcgccgtgaactccaggggcgagtttaccggcacatacatcaccgccgtgaccgccacctccaacgagatcaaggagtcccccctgcacggcacccagaacaccatcaataagaggacccagcccacctttggctttaccgtgaattggaagttctccgagtccaccacagtgtttacaggccagtgttttatcgataggaatggcaaggaggtgctgaagaccatgtggctgctgagatccagcgtgaatgatatcggcgatgactggaaggccaccagagtgggcatcaatatctttacaaggctgagaacccagaaggagtaatag

SEQ ID NO: 3 - RNA, 21 nt, synthetic construct
  source 1..21: mol_type = other RNA
gacgtaaacggccacaagttt